European Patent Specification EP 4 526 289 B1, published July 8, 2026. Title: ANTIVIRAL INDOLINYL COMPOUNDS AND USES THEREOF. Applicant: Gilead Sciences, Inc. The sequence listing filed with the application follows.

SEQUENCE LISTING (3 sequences)

SEQ ID NO: 1 - DNA, 22 bp, synthetic construct
  source 1..22: mol_type = other DNA
agagggacatccaggactttgt

SEQ ID NO: 2 - DNA, 19 bp, synthetic construct
  source 1..19: mol_type = other DNA
caggcgcttgttggtgtac

SEQ ID NO: 3 - DNA, 16 bp, synthetic construct
  source 1..16: mol_type = other DNA
accgccgaactgagca